European Patent Application EP 4 722 370 A1, published April 8, 2026. Title: 用于治疗癌症的组合物及其应用. Applicant: 上海先博生物科技有限公司. The sequence listing filed with the application follows.

SEQUENCE LISTING (84 sequences)

SEQ ID NO: 1 - protein, 20 aa, synthetic construct
MALPVTALLPLALLLHAARP

SEQ ID NO: 2 - protein, 45 aa, synthetic construct
TTTPAPRPPTPAPTIASQPLSLRPEACRPAAGGAVHTRGLDFACD

SEQ ID NO: 3 - protein, 40 aa, synthetic construct
IEVMYPPPYLDNEKSNGTIIHVKGKHLCPPSPLFPGPSKP

SEQ ID NO: 4 - protein, 24 aa, synthetic construct
IYIWAPLAGTCGVLLLSLVITLYC

SEQ ID NO: 5 - protein, 27 aa, synthetic construct
FWVLVVVGGVLACYSLLVTVAFIIFWV

SEQ ID NO: 6 - protein, 42 aa, synthetic construct
KRGRKKLLYIFKQPFMRPVQTTQEEDGCSCRFPEEEEGGCEL

SEQ ID NO: 7 - protein, 65 aa, synthetic construct
LVVVGGVLACYSLLVTVAFIIFWVRSKRSRLLHSDYMNMTPRRPGPTRKHYQPYAPPRDFAAYRS

SEQ ID NO: 8 - protein, 112 aa, synthetic construct
RVKFSRSADAPAYQQGQNQLYNELNLGRREEYDVLDKRRGRDPEMGGKPRRKNPQEGLYNELQKDKMAEAYSEIGMKGERRRGKGHDGLYQGLSTATKDTYDALHMQALPPR

SEQ ID NO: 9 - protein, 18 aa, synthetic construct
EGRGSLLTCGDVEENPGP

SEQ ID NO: 10 - protein, 19 aa, synthetic construct
ATNFSLLKQAGDVEENPGP

SEQ ID NO: 11 - protein, 15 aa, synthetic construct
GGGGSGGGGSGGGGS

SEQ ID NO: 12 - protein, 20 aa, synthetic construct
GGGGSGGGGSGGGGSGGGGS

SEQ ID NO: 13 - protein, 240 aa, synthetic construct
DIVMTQSPLSLPVTPGEPASISCRASQTISDYLHWYLQKPGQSPQLLIKYASQSISGVPDRFSGSGSGSDFTLKISRVEAEDVGVYYCQQGHSFPLTFGQGTKLEIKGGGGSGGGGSGGGGSEVQLVQSGAEVKKPGASVKVSCKASGYTFTSYWMHWVRQAPGQRLEWMGTIYPGNSDTRYNQKFKDRVTITADTSASTAYMELSSLRSEDTAVYYCTRSYDYGDLDYWGQGTTVTVSS

SEQ ID NO: 14 - protein, 118 aa, synthetic construct
EVQLVQSGAEVKKPGASVKVSCKASGYTFTSYWMHWVRQAPGQRLEWMGTIYPGNSDTRYNQKFKDRVTITADTSASTAYMELSSLRSEDTAVYYCTRSYDYGDLDYWGQGTTVTVSS

SEQ ID NO: 15 - protein, 107 aa, synthetic construct
DIVMTQSPLSLPVTPGEPASISCRASQTISDYLHWYLQKPGQSPQLLIKYASQSISGVPDRFSGSGSGSDFTLKISRVEAEDVGVYYCQQGHSFPLTFGQGTKLEIK

SEQ ID NO: 16 - protein, 5 aa, synthetic construct
SYWMH

SEQ ID NO: 17 - protein, 17 aa, synthetic construct
TIYPGNSDTRYNQKFKD

SEQ ID NO: 18 - protein, 9 aa, synthetic construct
SYDYGDLDY

SEQ ID NO: 19 - protein, 11 aa, synthetic construct
RASQTISDYLH

SEQ ID NO: 20 - protein, 7 aa, synthetic construct
YASQSIS

SEQ ID NO: 21 - protein, 9 aa, synthetic construct
QQGHSFPLT

SEQ ID NO: 22 - protein, 155 aa, synthetic construct
QRFAQAQQQLPLESLGWDVAELQLNHTGPQQDPRLYWQGGPALGRSFLHGPELDKGQLRIHRDGIYMVHIQVTLAICSSTTASRHHPTTLAVGICSPASRSISLLRLSFHQGCTIASQRLTPLARGDTLCTNLTGTLLPSRNTDETFFGVQWVRP

SEQ ID NO: 23 - protein, 193 aa, synthetic construct
MPEEGSGCSVRRRPYGCVLRAALVPLVAGLVICLVVCIQRFAQAQQQLPLESLGWDVAELQLNHTGPQQDPRLYWQGGPALGRSFLHGPELDKGQLRIHRDGIYMVHIQVTLAICSSTTASRHHPTTLAVGICSPASRSISLLRLSFHQGCTIASQRLTPLARGDTLCTNLTGTLLPSRNTDETFFGVQWVRP

SEQ ID NO: 24 - protein, 483 aa, synthetic construct
MALPVTALLLPLALLLHAARPDIVMTQSPLSLPVTPGEPASISCRASQTISDYLHWYLQKPGQSPQLLIKYASQSISGVPDRFSGSGSGSDFTLKISRVEAEDVGVYYCQQGHSFPLTFGQGTKLEIKGGGGSGGGGSGGGGSEVQLVQSGAEVKKPGASVKVSCKASGYTFTSYWMHWVRQAPGQRLEWMGTIYPGNSDTRYNQKFKDRVTITADTSASTAYMELSSLRSEDTAVYYCTRSYDYGDLDYWGQGTTVTVSSAAAIEVMYPPPYLDNEKSNGTIIHVKGKHLCPSPLFPGPSKPFWVLVVVGGVLACYSLLVTVAFIIFWVRSKRSRLLHSDYMNMTPRRPGPTRKHYQPYAPPRDFAAYRSRVKFSRSADAPAYQQGQNQLYNELNLGRREEYDVLDKRRGRDPEMGGKPRRKNPQEGLYNELQKDKMAEAYSEIGMKGERRRGKGHDGLYQGLSTATKDTYDALHMQALPPR

SEQ ID NO: 25 - protein, 686 aa, synthetic construct
MALPVTALLLPLALLLHAARPDIVMTQSPLSLPVTPGEPASISCRASQTISDYLHWYLQKPGQSPQLLIKYASQSISGVPDRFSGSGSGSDFTLKISRVEAEDVGVYYCQQGHSFPLTFGQGTKLEIKGGGGSGGGGSGGGGSEVQLVQSGAEVKKPGASVKVSCKASGYTFTSYWMHWVRQAPGQRLEWMGTIYPGNSDTRYNQKFKDRVTITADTSASTAYMELSSLRSEDTAVYYCTRSYDYGDLDYWGQGTTVTVSSTTTPAPRPPTPAPTIASQPLSLRPEACRPAAGGAVHTRGLDFACDIYIWAPLAGTCGVLLLSLVITLYCKRGRKKLLYIFKQPFMRPVQTTQEEDGCSCRFPEEEEGGCELRVKFSRSADAPAYQQGQNQLYNELNLGRREEYDVLDKRRGRDPEMGGKPRRKNPQEGLYNELQKDKMAEAYSEIGMKGERRRGKGHDGLYQGLSTATKDTYDALHMQALPPRKRRSGSGATNFSLLKQAGDVEENPGPMALPVTALLLPLALLLHAARPQRFAQAQQQLPLESLGWDVAELQLNHTGPQQDPRLYWQGGPALGRSFLHGPELDKGQLRIHRDGIYMVHIQVTLAICSSTTASRHHPTTLAVGICSPASRSISLLRLSFHQGCTIASQRLTPLARGDTLCTNLTGTLLPSRNTDETFFGVQWVRP

SEQ ID NO: 26 - protein, 703 aa, synthetic construct
MALPVTALLLPLALLLHAARPDIVMTQSPLSLPVTPGEPASISCRASQTISDYLHWYLQKPGQSPQLLIKYASQSISGVPDRFSGSGSGSDFTLKISRVEAEDVGVYYCQQGHSFPLTFGQGTKLEIKGGGGSGGGGSGGGGSEVQLVQSGAEVKKPGASVKVSCKASGYTFTSYWMHWVRQAPGQRLEWMGTIYPGNSDTRYNQKFKDRVTITADTSASTAYMELSSLRSEDTAVYYCTRSYDYGDLDYWGQGTTVTVSSTTTPAPRPPTPAPTIASQPLSLRPEACRPAAGGAVHTRGLDFACDIYIWAPLAGTCGVLLLSLVITLYCKRGRKKLLYIFKQPFMRPVQTTQEEDGCSCRFPEEEEGGCELRVKFSRSADAPAYQQGQNQLYNELNLGRREEYDVLDKRRGRDPEMGGKPRRKNPQEGLYNELQKDKMAEAYSEIGMKGERRRGKGHDGLYQGLSTATKDTYDALHMQALPPRKRRSGSGATNFSLLKQAGDVEENPGPMPEEGSGCSVRRRPYGCVLRAALVPLVAGLVICLVVCIQRFAQAQQQLPLESLGWDVAELQLNHTGPQQDPRLYWQGGPALGRSFLHGPELDKGQLRIHRDGIYMVHIQVTLAICSSTTASRHHPTTLAVGICSPASRSISLLRLSFHQGCTIASQRLTPLARGDTLCTNLTGTLLPSRNTDETFFGVQWVRP

SEQ ID NO: 27 - protein, 246 aa, synthetic construct
QVQLVQSGAEVKKPGSSVKVSCKASGYAFSNYLIEWVKQAPGQGLEWIGLINPGSGGTNYNEKFKGKATITADKSTSTAYMELSSLRSEDTAVYYCARVYYGNSFAYWGQGTLVTVSSGGGGSGGGGSGGGGSDIVMTQSPDSLAVSLGERATISCKSSQSLLNSGNQKNYLTWYQQKPGQPPKLLIYWASTRESGVPDRFSGSGSGTDFTLTISSLQAEDVAVYYCQNDYFYPFTFGQGTKLEIK

SEQ ID NO: 28 - protein, 118 aa, synthetic construct
QVQLVQSGAEVKKPGSSVKVSCKASGYAFSNYLIEWVKQAPGQGLEWIGLINPGSGGTNYNEKFKGKATITADKSTSTAYMELSSLRSEDTAVYYCARVYYGNSFAYWGQGTLVTVSS

SEQ ID NO: 29 - protein, 113 aa, synthetic construct
DIVMTQSPDSLAVSLGERATISCKSSQSLLNSGNQKNYLTWYQQKPGQPPKLLIYWASTRESGVPDRFSGSGSGTDFTLTISSLQAEDVAVYYCQNDYFYPFTFGQGTKLEIK

SEQ ID NO: 30 - protein, 5 aa, synthetic construct
NYLIE

SEQ ID NO: 31 - protein, 17 aa, synthetic construct
LINPGSGGTNYNEKFKG

SEQ ID NO: 32 - protein, 9 aa, synthetic construct
VYYGNSFAY

SEQ ID NO: 33 - protein, 17 aa, synthetic construct
KSSQSLLNSGNQKNYLT

SEQ ID NO: 34 - protein, 7 aa, synthetic construct
WASTRES

SEQ ID NO: 35 - protein, 9 aa, synthetic construct
QNDYFYPFT

SEQ ID NO: 36 - protein, 489 aa, synthetic construct
MALPVTALLLPLALLLHAARPQVQLVQSGAEVKKPGSSVKVSCKASGYAFSNYLIEWVKQAPGQGLEWIGLINPGSGGTNYNEKFKGKATITADKSTSTAYMELSSLRSEDTAVYYCARVYYGNSFAYWGQGTLVTVSSGGGGSGGGGSGGGGSDIVMTQSPDSLAVSLGERATISCKSSQSLLNSGNQKNYLTWYQQKPGQPPKLLIYWASTRESGVPDRFSGSGSGTDFTLTISSLQAEDVAVYYCQNDYFYPFTFGQGTKLEIKAAAIEVMYPPPYLDNEKSNGTIIHVKGKHLCPSPLFPGPSKPFWVLVVVGGVLACYSLLVTVAFIIFWVRSKRSRLLHSDYMNMTPRRPGPTRKHYQPYAPPRDFAAYRSRVKFSRSADAPAYQQGQNQLYNELNLGRREEYDVLDKRRGRDPEMGGKPRRKNPQEGLYNELQKDKMAEAYSEIGMKGERRRGKGHDGLYQGLSTATKDTYDALHMQALPPR

SEQ ID NO: 37 - protein, 691 aa, synthetic construct
MALPVTALLLPLALLLHAARPQVQLVQSGAEVKKPGSSVKVSCKASGYAFSNYLIEWVKQAPGQGLEWIGLINPGSGGTNYNEKFKGKATITADKSTSTAYMELSSLRSEDTAVYYCARVYYGNSFAYWGQGTLVTVSSGGGGSGGGGSGGGGSDIVMTQSPDSLAVSLGERATISCKSSQSLLNSGNQKNYLTWYQQKPGQPPKLLIYWASTRESGVPDRFSGSGSGTDFTLTISSLQAEDVAVYYCQNDYFYPFTFGQGTKLEIKAAAIEVMYPPPYLDNEKSNGTIIHVKGKHLCPSPLFPGPSKPFWVLVVVGGVLACYSLLVTVAFIIFWVRSKRSRLLHSDYMNMTPRRPGPTRKHYQPYAPPRDFAAYRSRVKFSRSADAPAYQQGQNQLYNELNLGRREEYDVLDKRRGRDPEMGGKPRRKNPQEGLYNELQKDKMAEAYSEIGMKGERRRGKGHDGLYQGLSTATKDTYDALHMQALPPRKRRSGSGATNFSLLKQAGDVEENPGPMALPVTALLLPLALLLHAARPQRFAQAQQQLPLESLGWDVAELQLNHTGPQQDPRLYWQGGPALGRSFLHGPELDKGQLRIHRDGIYMVHIQVTLAICSSTTASRHHPTTLAVGICSPASRSISLLRLSFHQGCTIASQRLTPLARGDTLCTNLTGTLLPSRNTDETFFGVQWVRP

SEQ ID NO: 38 - protein, 708 aa, synthetic construct
MALPVTALLLPLALLLHAARPQVQLVQSGAEVKKPGSSVKVSCKASGYAFSNYLIEWVKQAPGQGLEWIGLINPGSGGTNYNEKFKGKATITADKSTSTAYMELSSLRSEDTAVYYCARVYYGNSFAYWGQGTLVTVSSGGGGSGGGGSGGGGSDIVMTQSPDSLAVSLGERATISCKSSQSLLNSGNQKNYLTWYQQKPGQPPKLLIYWASTRESGVPDRFSGSGSGTDFTLTISSLQAEDVAVYYCQNDYFYPFTFGQGTKLEIKAAAIEVMYPPPYLDNEKSNGTIIHVKGKHLCPSPLFPGPSKPFWVLVVVGGVLACYSLLVTVAFIIFWVRSKRSRLLHSDYMNMTPRRPGPTRKHYQPYAPPRDFAAYRSRVKFSRSADAPAYQQGQNQLYNELNLGRREEYDVLDKRRGRDPEMGGKPRRKNPQEGLYNELQKDKMAEAYSEIGMKGERRRGKGHDGLYQGLSTATKDTYDALHMQALPPRKRRSGSGATNFSLLKQAGDVEENPGPMPEEGSGCSVRRRPYGCVLRAALVPLVAGLVICLVVCIQRFAQAQQQLPLESLGWDVAELQLNHTGPQQDPRLYWQGGPALGRSFLHGPELDKGQLRIHRDGIYMVHIQVTLAICSSTTASRHHPTTLAVGICSPASRSISLLRLSFHQGCTIASQRLTPLARGDTLCTNLTGTLLPSRNTDETFFGVQWVRP

SEQ ID NO: 39 - protein, 121 aa, synthetic construct
EVQLVESGGGLVKPGGSLRLSCAASGRTSTIHRMGWFRQAPGKEREFVSSISRVSSTTYYADSVKGRFTISRDNAKNSLYLQMNSLRAEDTAVYYCAASEYEVSPGKSKYWGQGTMVTVSS

SEQ ID NO: 40 - protein, 5 aa, synthetic construct
IHRMG

SEQ ID NO: 41 - protein, 17 aa, synthetic construct
SISRVSSTTYYADSVKG

SEQ ID NO: 42 - protein, 12 aa, synthetic construct
SEYEVSPGKSKY

SEQ ID NO: 43 - protein, 364 aa, synthetic construct
MALPVTALLLPLALLLHAARPEVQLVESGGGLVKPGGSLRLSCAASGRTSTIHRMGWFRQAPGKEREFVSSISRVSSTTYYADSVKGRFTISRDNAKNSLYLQMNSLRAEDTAVYYCAASEYEVSPGKSKYWGQGTMVTVSSAAAIEVMYPPPYLDNEKSNGTIIHVKGKHLCPSPLFPGPSKPFWVLVVVGGVLACYSLLVTVAFIIFWVRSKRSRLLHSDYMNMTPRRPGPTRKHYQPYAPPRDFAAYRSRVKFSRSADAPAYQQGQNQLYNELNLGRREEYDVLDKRRGRDPEMGGKPRRKNPQEGLYNELQKDKMAEAYSEIGMKGERRRGKGHDGLYQGLSTATKDTYDALHMQALPPR

SEQ ID NO: 44 - protein, 566 aa, synthetic construct
MALPVTALLLPLALLLHAARPEVQLVESGGGLVKPGGSLRLSCAASGRTSTIHRMGWFRQAPGKEREFVSSISRVSSTTYYADSVKGRFTISRDNAKNSLYLQMNSLRAEDTAVYYCAASEYEVSPGKSKYWGQGTMVTVSSAAAIEVMYPPPYLDNEKSNGTIIHVKGKHLCPSPLFPGPSKPFWVLVVVGGVLACYSLLVTVAFIIFWVRSKRSRLLHSDYMNMTPRRPGPTRKHYQPYAPPRDFAAYRSRVKFSRSADAPAYQQGQNQLYNELNLGRREEYDVLDKRRGRDPEMGGKPRRKNPQEGLYNELQKDKMAEAYSEIGMKGERRRGKGHDGLYQGLSTATKDTYDALHMQALPPRKRRSGSGATNFSLLKQAGDVEENPGPMALPVTALLLPLALLLHAARPQRFAQAQQQLPLESLGWDVAELQLNHTGPQQDPRLYWQGGPALGRSFLHGPELDKGQLRIHRDGIYMVHIQVTLAICSSTTASRHHPTTLAVGICSPASRSISLLRLSFHQGCTIASQRLTPLARGDTLCTNLTGTLLPSRNTDETFFGVQWVRP

SEQ ID NO: 45 - protein, 583 aa, synthetic construct
MALPVTALLLPLALLLHAARPEVQLVESGGGLVKPGGSLRLSCAASGRTSTIHRMGWFRQAPGKEREFVSSISRVSSTTYYADSVKGRFTISRDNAKNSLYLQMNSLRAEDTAVYYCAASEYEVSPGKSKYWGQGTMVTVSSAAAIEVMYPPPYLDNEKSNGTIIHVKGKHLCPSPLFPGPSKPFWVLVVVGGVLACYSLLVTVAFIIFWVRSKRSRLLHSDYMNMTPRRPGPTRKHYQPYAPPRDFAAYRSRVKFSRSADAPAYQQGQNQLYNELNLGRREEYDVLDKRRGRDPEMGGKPRRKNPQEGLYNELQKDKMAEAYSEIGMKGERRRGKGHDGLYQGLSTATKDTYDALHMQALPPRKRRSGSGATNFSLLKQAGDVEENPGPMPEEGSGCSVRRRPYGCVLRAALVPLVAGLVICLVVCIQRFAQAQQQLPLESLGWDVAELQLNHTGPQQDPRLYWQGGPALGRSFLHGPELDKGQLRIHRDGIYMVHIQVTLAICSSTTASRHHPTTLAVGICSPASRSISLLRLSFHQGCTIASQRLTPLARGDTLCTNLTGTLLPSRNTDETFFGVQWVRP

SEQ ID NO: 46 - protein, 208 aa, synthetic construct
MPEEGSGCSVRRRPYGCVLRAALVPLVAGLVICLVVCIQRFAQAQQQLPLESLGWDVAELQLNHTGPQQDPRLYWQGGPALGRSFLHGPELDKGQLRIHRDGIYMVHIQVTLAICSSTTASRHHPTTLAVGICSPASRSISLLRLSFHQGLFGFWNWGLKVKCFLRHLIWTAHCFIPLTQLVFMQALQSWRNHHCSHFTDEENRGVNR

SEQ ID NO: 47 - protein, 170 aa, synthetic construct
QRFAQAQQQLPLESLGWDVAELQLNHTGPQQDPRLYWQGGPALGRSFLHGPELDKGQLRIHRDGIYMVHIQVTLAICSSTTASRHHPTTLAVGICSPASRSISLLRLSFHQGLFGFWNWGLKVKCFLRHLIWTAHCFIPLTQLVFMQALQSWRNHHCSHFTDEENRGVNR

SEQ ID NO: 48 - protein, 244 aa, synthetic construct
DIVMTQSQKFMSTSVGDRVSITCKASQNVGTAVAWYQQKPGQSPKLLIFSASIRYTGVPDRFTGSGSGTDFTLTISNMQSEDLADYFCQQYSSSPYTFGGGTKLEIKGGGGSGGGGSGGGGSEVQLQQSGPVLVKPGASVKMSCKASGYTFTDYYMNWVKRSHGKSLEWIGIINPYNGGTSYNQKFRGKATLTVDKSSNTAYMELNSLTSEDSAVYYCSRYDYDYDVEGAMDYWGQGTSVTVSS

SEQ ID NO: 49 - protein, 240 aa, synthetic construct
DIVMTQSPATLSVTPGDRVSLSCRASQTISDYLHWYQQRSHESPRLLIKYASQSISGIPSRFSGSGSGSDFTLSINSVEPEDVGVYYCQNGHSFPLTFGAGTKLELKGGGGSGGGGSGGGGSEVQLQQSGTVLARPGASVKMSCKTSGYTFTSYWMHWVKQSPGQGLEWIGTIYPGNSDTRYNQKFKDKAYVTAVTSASTAYMELSSLTNEESAVYYCTRSYDYGDLDYWGQGTTLTVSS

SEQ ID NO: 50 - protein, 245 aa, synthetic construct
DIVLTQSPASLAVSLGQRATISCRASKSVSTSGFSYMHWYQQKPGQPPKLLIYLASNLESGVPARFSGSGSGTDFTLNIHPVEEEDAATYYCQHSRELPFTFGSGTKLEIKGGGGSGGGGSGGGGSQVQLQQSGAELVKPGASVRISCKASGYAFSNYWINWVKQRPGKGLEWIGQINPGDGDTIYNGKFKGKATLTADKSSSTAYMQLSSLTSEDSAVYFCEREGRNYGDFAYWGQGTTLTVSS

SEQ ID NO: 51 - protein, 246 aa, synthetic construct
DIVMTQSPDSLAVSLGERATISCKSSQSLLNSGNQKNYLTWYQQKPGQPPKLLIYWASTRESGVPDRFSGSGSGTDFTLTISSLQAEDVAVYYCQNDYFYPFTFGQGTKLEIKGGGGSGGGGSGGGGSQVQLVQSGAEVKKPGSSVKVSCKASGYAFSNYLIEWVKQAPGQGLEWIGLINPGSGGTNYNEKFKGKATITADKSTSTAYMELSSLRSEDTAVYYCARVYYGNSFAYWGQGTLVTVSS

SEQ ID NO: 52 - protein, 246 aa, synthetic construct
DIVMTQSPDSLAVSLGERATINCKSSQSLFNSGNQKNYLTWYQQKPGQPPKLLIYWASTRESGVPDRFSGSGSGTDFTLTISSLQAEDVAVYYCQNAYSFPYTFGGGTKLEIKGGGGSGGGGSGGGGSQVQLQESGPGLIKPSQTLSLTCTVSGGSISSGYNWHWIRQPPGKGLEWIGYIHYTGSTNYNPALRSRVTISVDTSKNQFSLKLSSVTAADTAIYYCARIYNGNSFPYWGQGTTVTVSS

SEQ ID NO: 53 - protein, 129 aa, synthetic construct
EVQLVESGGGLVQPGRSLRLSCAASVLNLDYYAITWFRQAPGKEREGVSCIQGRGTSTNYADSVKGRFTISRDRAKKSAYLQMNSLRAEDTALYYCAVRYVSYGRNTACGLLPESVDHWGQGTMVTVSS

SEQ ID NO: 54 - protein, 123 aa, synthetic construct
EVQLVESGGGLVQPGGSLRLSCAASGFTLDDYAIGWFRQAPGKEREGVICLTSGGLPKYADSVKGRFTISRDNSKNTLYLQMNSLRAEDTAVYYCAASGATSRWNCPPQYDHWGQGTMVTVSS

SEQ ID NO: 55 - protein, 5 aa, synthetic construct
GGGGS

SEQ ID NO: 56 - protein, 10 aa, synthetic construct
GGGGSGGGGS

SEQ ID NO: 57 - protein, 18 aa, synthetic construct
GSTSGSGKPGSGEGSTKG

SEQ ID NO: 58 - protein, 22 aa, synthetic construct
MVLLVTSLLLCELPHPAFLLIP

SEQ ID NO: 59 - protein, 19 aa, synthetic construct
MEFGLSWVFLVALLRGVQC

SEQ ID NO: 60 - protein, 112 aa, synthetic construct
RVKFSRSADAPAYKQGQNQLYNELNLGRREEYDVLDKRRGRDPEMGGKPRRKNPQEGLYNELQKDKMAEAYSEIGMKGERRRGKGHDGLYQGLSTATKDTYDALHMQALPPR

SEQ ID NO: 61 - DNA, 213 bp, synthetic construct
  source 1..213: mol_type = other DNA
gggcagagcgcacatcgcccacagtccccgagaagttggggggaggggtcggcaattgaaccggtgcctagagaaggtggcgcggggtaaactgggaaagtgatgtcgtgtactggctccgccttttttcccgagggtgggggagaaccgtatataagtgcagtagtcgccgtgaacgttctttttcgcaacgggtttgccgccagaacacag

SEQ ID NO: 62 - DNA, 535 bp, synthetic construct
  source 1..535: mol_type = other DNA
tcgattagtccaatttgttaaagacaggatatcagtggtccaggctctagttttgactcaacaatatcaccagctgaagcctatagagtacgagccatagatagaataaaagattttatttagtctccagaaaaaggggggaatgaaagaccccacctgtaggtttggcaagctaggatcaaggttaggaacagagagacagcagaatatgggccaaacaggatatctgtggtaagcagttcctgccccggctcagggccaagaacagttggaacagcagaatatgggccaaacaggatatctgtggtaagcagttcctgccccggctcagggccaagaacagatggtccccagatgcggtcccgccctcagcagtttctagagaaccatcagatgtttccagggtgccccaaggacctgaaatgaccctgtgccttatttgaactaaccaatcagttcgcttctcgcttctgttcgcgcgcttctgctccccgagctcaataaaagagcccacaacccctcactcggcgcgatc

SEQ ID NO: 63 - protein, 693 aa, synthetic construct
MALPVTALLLPLALLLHAARPDVVMTQSPLSLPVTPGEPASISCRSSQSLVHSNANTYLHWYLQKPGQSPQLLIYKVSNRFSGVPDRFSGSGSGTDFTLKISRVEAEDVGVYYCSQNTHVPPTFGQGTKLEIKRGGGGSGGGGSGGGGSQVQLVQSGAEVKKPGASVKVSCKASGYTFTDYEMHWVRQAPGQGLEWMGALDPKTGDTAYSQKFKGRVTLTADESTSTAYMELSSLRSEDTAVYYCTRFYSYTYWGQGTLVTVSSASTTTPAPRPPTPAPTIASQPLSLRPEACRPAAGGAVHTRGLDFACDIYIWAPLAGTCGVLLLSLVITLYCKRGRKKLLYIFKQPFMRPVQTTQEEDGCSCRFPEEEEGGCELRVKFSRSADAPAYKQGQNQLYNELNLGRREEYDVLDKRRGRDPEMGGKPRRKNPQEGLYNELQKDKMAEAYSEIGMKGERRRGKGHDGLYQGLSTATKDTYDALHMQALPPRKRRSGSGATNFSLLKQAGDVEENPGPMALPVTALLLPLALLLHAARPGGQRFAQAQQQLPLESLGWDVAELQLNHTGPQQDPRLYWQGGPALGRSFLHGPELDKGQLRIHRDGIYMVHIQVTLAICSSTTASRHHPTTLAVGICSPASRSISLLRLSFHQGCTIASQRLTPLARGDTLCTNLTGTLLPSRNTDETFFGVQWVRP

SEQ ID NO: 64 - protein, 243 aa, synthetic construct
DVVMTQSPLSLPVTPGEPASISCRSSQSLVHSNANTYLHWYLQKPGQSPQLLIYKVSNRFSGVPDRFSGSGSGTDFTLKISRVEAEDVGVYYCSQNTHVPPTFGQGTKLEIKRGGGGSGGGGSGGGGSQVQLVQSGAEVKKPGASVKVSCKASGYTFTDYEMHWVRQAPGQGLEWMGALDPKTGDTAYSQKFKGRVTLTADESTSTAYMELSSLRSEDTAVYYCTRFYSYTYWGQGTLVTVSS

SEQ ID NO: 65 - protein, 122 aa, synthetic construct
QVQLVESGGGLVQPGGSLRLSCAASGSISTYTMAWYRQAPGEQRESVAAISSGGRTDYIDSVKGRFTISRDNAKNMVYLQMNSLKPEDTAVYYCNSADGLKIGTYYFKGLGWGQGTQVTVSA

SEQ ID NO: 66 - protein, 123 aa, synthetic construct
QLQLVESGGGLVQPGGSLRLSCAASGFTLDVYAIGWFRQAPGKEREGVSYITSGDGIFYADSVKGRFTISRDNAKNTVYLQMNSLKPEDTAVYFCATLKRTTAGGWPIPGRIGGQGTQVTVSS

SEQ ID NO: 67 - protein, 124 aa, synthetic construct
QVQLVESGGGLVQPGGSLRLSCAASGFTLDAYAIGWFRQAPGKEREGVSYITSGTGTTLYADSVKGRFTISRDNAKNTVYLQMNSLKPEDTAVYFCTTLKRTTAGGWPIPGRIGGQGTQVTVSS

SEQ ID NO: 68 - protein, 124 aa, synthetic construct
QVQLVESGGGLVQAGGSLRLSCAASGFTLENYAIGWFRQAPGKEREGVSYITGGTGTTVYADSVKGRFTISRDNTKNTVYLQMNSLKPEDTAVYFCATLKRTTAGGWPKPGRIGGQGTQVTVSS

SEQ ID NO: 69 - protein, 124 aa, synthetic construct
QLQLVESGGGLVQPGGSLRLSCAASGFTLDVYAIGWFRQAPGKEREGVSYITGGTGTTVYADSVKGRFTISRDNTKNTVYLQMNSLKPEDTAVYFCATLKRTTAGGWPKPGRIGGQGTQVTVSS

SEQ ID NO: 70 - protein, 124 aa, synthetic construct
QVQLVESGGGLVQAGGSLSLSCAASGRRFSTNVMGWFRQAPGKEREFLAAINWVIGNTNYAESVKGRFTISRDNAKETVYLQMDNLKVEDTAVYYCAGRSSYYTSSRREDYDYWGQGTQVTVSS

SEQ ID NO: 71 - protein, 120 aa, synthetic construct
QVQLVESGGGLVQLGGSLTLSCVASGDVHKINAKGWYRQAPGKEREVVAIITSGGTPYYADAVKGRFTISRHDDKNTVTLQMNSLKPEDTAMYYCAAGLRGMGPYDYDYRGPGTQVTVSS

SEQ ID NO: 72 - protein, 123 aa, synthetic construct
QVQLVESGGGLVQAGGSLKLSCAASGRSFSPYAMGWFRQAPGKDREFVAAISNSGGSTYYADAVKGRFSISRDNAKNTVYLQMNNLEPEDTAVYYCTGPVKRYSTDFQGGDYWGQGTQVTVSS

SEQ ID NO: 73 - protein, 123 aa, synthetic construct
QVQLVESGGGLVQAGGSLRLSCAFSGRTFSKYAMAWFRQAPGKGRDFVARVGPSGRTTDYADSVKGRFTVSRDNAKNTVSLQMSSLKPDDAALYYCAATSGIYGESYNLYNYWGQGTQVTVSS

SEQ ID NO: 74 - protein, 123 aa, synthetic construct
QVQLVESGGGLVRPGGSLRVSCAASGVDISTYTMAWYRQAPGEQRESVAAISTTGRSIYIDAVQGRFTMSRDNAKNTVYLQMNNLKPEDTAVYYCNSADDLKIGTQYFKGLGWGQGTQVTVSS

SEQ ID NO: 75 - protein, 123 aa, synthetic construct
QVQLVESGGGLVQAGASLRLSCLGSGRSFGLRAMGWFRQAPGKELEFVAAIGKAGDTTYYTDSVKGRFTISRDNVKNAVYLQMNSLKPEDTAVYVCATAARWEPPTITPGSYRGPGTQVTVSS

SEQ ID NO: 76 - protein, 115 aa, synthetic construct
QVQLVQSGAEVKKPGASVKVSCKASGYTFTDYEMHWVRQAPGQGLEWMGALDPKTGDTAYSQKFKGRVTLTADESTSTAYMELSSLRSEDTAVYYCTRFYSYTYWGQGTLVTVSS

SEQ ID NO: 77 - protein, 536 aa, synthetic construct
MALPVTALLLPLALLLHAARPDVVMTQSPLSLPVTPGEPASISCRSSQSLVHSNANTYLHWYLQKPGQSPQLLIYKVSNRFSGVPDRFSGSGSGTDFTLKISRVEAEDVGVYYCSQNTHVPPTFGQGTKLEIKRGGGGSGGGGSGGGGSQVQLVQSGAEVKKPGASVKVSCKASGYTFTDYEMHWVRQAPGQGLEWMGALDPKTGDTAYSQKFKGRVTLTADESTSTAYMELSSLRSEDTAVYYCTRFYSYTYWGQGTLVTVSSASTTTPAPRPPTPAPTIASQPLSLRPEACRPAAGGAVHTRGLDFACDIYIWAPLAGTCGVLLLSLVITLYCKRGRKKLLYIFKQPFMRPVQTTQEEDGCSCRFPEEEEGGCELRVKFSRSADAPAYKQGQNQLYNELNLGRREEYDVLDKRRGRDPEMGGKPRRKNPQEGLYNELQKDKMAEAYSEIGMKGERRRGKGHDGLYQGLSTATKDTYDALHMQALPPRKRRSGSGATNFSLLKQAGDVEENPGPMALPVTALLLPLALLLHAARP

SEQ ID NO: 78 - protein, 22 aa, synthetic construct
GSGATNFSLLKQAGDVEENPGP

SEQ ID NO: 79 - protein, 21 aa, synthetic construct
GSGEGRGSLLTCGDVEENPGP

SEQ ID NO: 80 - protein, 23 aa, synthetic construct
GSGQCTNYALLKLAGDVESNPGP

SEQ ID NO: 81 - protein, 20 aa, synthetic construct
QCTNYALLKLAGDVESNPGP

SEQ ID NO: 82 - protein, 25 aa, synthetic construct
GSGVKQTLNFDLLKLAGDVESNPGP

SEQ ID NO: 83 - protein, 22 aa, synthetic construct
VKQTLNFDLLKLAGDVESNPGP

SEQ ID NO: 84 - protein, 20 aa, synthetic construct
TRAEIEDELIRRGIESNPGP